European Patent Application EP 4 112 067 A1, published January 4, 2023. Title: 锰型高稳定性超氧化物歧化酶在脑卒中预防或治疗中的应用. Applicant: 凯睿恒济生物医药（杭州）有限公司. The sequence listing filed with the application follows.

SEQUENCE LISTING (4 sequences)

SEQ ID NO: 1 - DNA, 28 bp, 人工序列(Artificial Sequence)
aagaattcatgccgtacccgttcaagct

SEQ ID NO: 2 - DNA, 27 bp, 人工序列(Artificial Sequence)
ctgtcgactcaggctttgttgaagaac

SEQ ID NO: 3 - DNA, 615 bp, 人工序列(Artificial Sequence)
atgccgtacccgttcaagcttcctgacctaggctacccctacgaggccctcgagccccacattgacgccaagaccatggagatccaccaccagaagcaccacggggcctacgtgacgaacctcaacgccgccctggagaagtacccctacctccacggggtggaggtggaggtcctcctgaggcacctcgccgcccttccccaggacatccagaccgccgtgcgcaacaacgggggcgggcacctgaaccacagcctcttctggaggctcctcacccccgggggggccaaggagcccgtgggggagctgaagaaggccattgacgagcagttcgggggcttccaggccctcaaggagaagctcacccaggcggccatgggccggttcggctcgggctgggcctggctcgtgaaggaccccttcggcaagctccacgtcctctccacccccaaccaagacaaccccgtgatggagggcttcacccccatcgtgggcattgacgtctgggagcacgcctactacctcaagtaccagaaccgccgggccgattacctccaggccatctggaacgtcctcaactgggacgtggccgaggagttcttcaataaagcctga

SEQ ID NO: 4 - protein, 204 aa, 人工序列(Artificial Sequence)
MPYPFKLPDLGYPYEALEPHIDAKTMEIHHQKHHGAYVTNLNAALEKYPYLHGVEVEVLLRHLAALPQDIQTAVRNNGGGHLNHSLFWRLLTPGGAKEPVGELKKAIDEQFGGFQALKEKLTQAAMGRFGSGWAWLVKDPFGKLHVLSTPNQDNPVMEGFTPIVGIDVWEHAYYLKYQNRRADYLQAIWNVLNWDVAEEFFKKA